European Patent Specification EP 3 551 188 B1, published October 18, 2023. Title: Substituted Quinazoline Sulfonamides as Thioredoxin Interacting Protein (TXNIP) Inhibitors. Applicant: The UAB Research Foundation Southern Research Institute Augelli-Szafran, Corinne E. Moukha-Chafiq, Omar Suto, Mark J. Shalev, Anath Thielen, Lance J. Chen, Junqin J. Jing, Gu J. The sequence listing filed with the application follows.

SEQUENCE LISTING (4 sequences)

SEQ ID NO: 1 - DNA, 20 bp, Artificial sequence
  Synthetic construct
cgagtcaaagccgtcaggat

SEQ ID NO: 2 - DNA, 24 bp, Artificial sequence
  Synthetic construct
ttcatagcgcaagtagtccaaggt

SEQ ID NO: 3 - DNA, 21 bp, Artificial sequence
  Synthetic construct
agtccctgccctttgtacaca

SEQ ID NO: 4 - DNA, 21 bp, Artificial sequence
  Synthetic construct
gatccgagggcctcactaaac